European Patent Specification EP 3 911 367 B1, published July 1, 2026. Title: THERAPEUTIC NANOCONJUGATES AND USES THEREOF. Applicant: UNIVERSITAT AUTÒNOMA DE BARCELONA FUNDACIÓ INSTITUT DE RECERCA DE L' HOSPITAL DE LA SANTA CREU I SANT PAU CENTRO DE INVESTIGACIÓN BIOMÉDICA EN RED. The sequence listing filed with the application follows.

SEQUENCE LISTING (36 sequences)

SEQ ID NO: 1 - protein, 9 aa, Artificial Sequence
  Polycationic peptide
RRRRRRRRR

SEQ ID NO: 2 - protein, 9 aa, Artificial Sequence
  Polycationic peptide
RRRGRGRRR

SEQ ID NO: 3 - protein, 9 aa, Artificial Sequence
  Polycationic peptide
RARGRGRRR

SEQ ID NO: 4 - protein, 9 aa, Artificial Sequence
  Polycationic peptide
RARGRGGGA

SEQ ID NO: 5 - protein, 18 aa, Artificial Sequence
  T22 peptide
RRWCYRKCYKGYCYRKCR

SEQ ID NO: 6 - protein, 21 aa, Artificial Sequence
  V1 peptide
LGASWHRPDKCCLGYQKRPLP

SEQ ID NO: 7 - protein, 67 aa, Artificial Sequence
  CXCL12 peptide
KPVSLSYRCPCRFFESHVARANVKHLKILNTPNCALQIVARLKNNNRQVCIDPKLKWIQEYLEKALN

SEQ ID NO: 8 - protein, 68 aa, Artificial Sequence
  vCCL2 peptide
LGASWHRPDKCCLGYQKRPLPQVLLSSWYPTSQLCSKPGVIFLTKRGRQVCADKDWVKKLMQQLPVTA

SEQ ID NO: 9 - protein, 14 aa, Artificial Sequence
  T140 peptide
  MISC_FEATURE (3)..(3): Xaa is L-3-(2-naphthyl)alanine
  MISC_FEATURE (8)..(8): Xaa is D-Lys
  MISC_FEATURE (12)..(12): Xaa is L-Citrulline
RRXCYRKXPYRXCR

SEQ ID NO: 10 - protein, 14 aa, Artificial Sequence
  TN14003 peptide
  MISC_FEATURE (3)..(3): Xaa is L-3-(2-naphthyl)alanine
  MISC_FEATURE (6)..(6): Xaa is L-Citrulline
  MISC_FEATURE (8)..(8): Xaa is D-Lys
  MISC_FEATURE (12)..(12): Xaa is L-Citrulline
RRXCYXKXPYRXCR

SEQ ID NO: 11 - protein, 14 aa, Artificial Sequence
  TC 14012 peptide
  MISC_FEATURE (3)..(3): Xaa is L-3-(2-naphthyl)alanine
  MISC_FEATURE (8)..(8): Xaa is D-Citrulline
  MISC_FEATURE (12)..(12): Xaa is L-Citrulline
RRXCYEKXPYRXCR

SEQ ID NO: 12 - protein, 14 aa, Artificial Sequence
  TE14011 peptide
  MISC_FEATURE (3)..(3): Xaa  is L-3-(2-naphthyl)alanine
  MISC_FEATURE (6)..(6): Xaa is  L-Citrulline
  MISC_FEATURE (8)..(8): Xaa is D-Glutamic acid
  MISC_FEATURE (12)..(12): Xaa is  L-Citrulline
RRXCYXKXPYRXCR

SEQ ID NO: 13 - protein, 14 aa, Artificial Sequence
  TZ14011 peptide
  MISC_FEATURE (3)..(3): Xaa is L-3-(2)-naphthyl)alanine
  MISC_FEATURE (6)..(6): Xaa is L-Citrulline
  MISC_FEATURE (8)..(8): Xaa is D-Lysine
  MISC_FEATURE (12)..(12): Xaa is L-Citrulline
RRXCYXKXPYRXCR

SEQ ID NO: 14 - protein, 20 aa, Artificial Sequence
  GW-H1 peptide
GYNYAKKLANLAKKFANALW

SEQ ID NO: 15 - protein, 13 aa, Artificial Sequence
  A5G27
RLVSYNGIIFFLK

SEQ ID NO: 16 - protein, 69 aa, Artificial Sequence
  FNI/II/V
WQPPRARITGYIIKYEKPGSPPREVVPRPRPGVTEATITGLEPGTEYTIYVIALKNNQKSEPLIGRKKT

SEQ ID NO: 17 - protein, 18 aa, Artificial Sequence
  Seq-1-7 peptide
KYLAYPDSVHIWRKRKRK

SEQ ID NO: 18 - protein, 19 aa, Artificial Sequence
  Seq-1-8 peptide
KYLAYPDSVHIWRKRKRKR

SEQ ID NO: 19 - protein, 22 aa, Artificial Sequence
  Angiopep-2-7 peptide
TFFYGGSRGKRNNFKTEEYRKR

SEQ ID NO: 20 - protein, 31 aa, Artificial Sequence
  Nucleolin binding peptide
KDEPQRRSARLSAKPAPPKPEPKPKKAPAKK

SEQ ID NO: 21 - protein, 39 aa, Artificial Sequence
  Nucleolin binding peptide
KDEPQRRSARLSAKPAPPKPEPKPKKAPAKKRKRKRKRK

SEQ ID NO: 22 - protein, 98 aa, Artificial sequence
  Stefin A
MIPGGLSEAKPATPEIQEIVDKVKPQLEEKTNETYGKLEAVQYKTQVVAGTNYYIKVRAGDNKYMHLKVFKSLPGQNEDLVLTGYQVDKNKDDELTGF

SEQ ID NO: 23 - protein, 14 aa, Artificial sequence
  Linker sequence
SGGTSGSTSGTGST

SEQ ID NO: 24 - protein, 15 aa, Artificial sequence
  Linker sequence
AGSSTGSSTGPGSTT

SEQ ID NO: 25 - protein, 7 aa, Artificial sequence
  Linker sequence
GGSGGAP

SEQ ID NO: 26 - protein, 8 aa, Artificial sequence
  Linker sequence
GGGVEGGG

SEQ ID NO: 27 - protein, 10 aa, Artificial sequence
  Linker sequence
PKPSTPPGSS

SEQ ID NO: 28 - protein, 11 aa, Artificial sequence
  Linker sequence
APAETKAEPMT

SEQ ID NO: 29 - protein, 5 aa, Artificial sequence
  Linker sequence
AAALE

SEQ ID NO: 30 - protein, 5 aa, Artificial sequence
  Protease cleavage site
DDDDK

SEQ ID NO: 31 - protein, 5 aa, Artificial sequence
  Protease cleavage site
IEDGR

SEQ ID NO: 32 - protein, 6 aa, Artificial sequence
  Protease cleavage site
LVPRGS

SEQ ID NO: 33 - protein, 7 aa, Artificial sequence
  Protease cleavage site
ENLYFQG

SEQ ID NO: 34 - protein, 8 aa, Artificial sequence
  Protease cleavage site
LEVLFQGP

SEQ ID NO: 35 - protein, 7 aa, Artificial sequence
  Linker sequence
GGSSRSS

SEQ ID NO: 36 - protein, 5 aa, Artificial sequence
  Linker sequence
GGGNS